European Patent Application EP 4 202 057 A1, published June 28, 2023. Title: DETECTION OF TELOMERE FUSION EVENTS. Applicant: European Molecular Biology Laboratory Centro Nacional de Investigaciones Cardiovasculares Carlos III F.S.P. (CNIC) CONSEJO SUPERIOR DE INVESTIGACIONES CIENTIFICAS (CSIC). The sequence listing filed with the application follows.

SEQUENCE LISTING (28 sequences)

SEQ ID NO: 1 - DNA, 16 bp, artificial
  oligonucleotide
gttagggttagggtta

SEQ ID NO: 2 - DNA, 18 bp, artificial
  oligonucleotide
ccctaaccctaaccctaa

SEQ ID NO: 3 - DNA, 20 bp, artificial
  oligonucleotide
ccctaaccctagggttaggg

SEQ ID NO: 4 - DNA, 21 bp, artificial
  oligonucleotide
ccctaacccttagggttaggg

SEQ ID NO: 5 - DNA, 16 bp, artificial
  oligonucleotide
ttagggttaaccctaa

SEQ ID NO: 6 - DNA, 15 bp, artificial
  oligonucleotide
ttagggtaaccctaa

SEQ ID NO: 7 - DNA, 28 bp, artificial
  oligonucleotide
ttagggttagggttagggttagggttag

SEQ ID NO: 8 - DNA, 18 bp, artificial
  oligonucleotide
ggctaaccctaaccctaa

SEQ ID NO: 9 - DNA, 32 bp, artificial
  oligonucleotide
ttagggttagggttagctaaccctaaccctaa

SEQ ID NO: 10 - DNA, 32 bp, artificial
  oligonucleotide
ccctaaccctaaccctagggttagggttaggg

SEQ ID NO: 11 - DNA, 58 bp, artificial
  oligonucleotide
ttagggttagggttagggttagggttagggttagggttagggttagggttagggttag

SEQ ID NO: 12 - DNA, 34 bp, artificial
  oligonucleotide
ctaaccctaaccctaaccctaaccctaaccctaa

SEQ ID NO: 13 - DNA, 57 bp, artificial
  oligonucleotide
ttagggttagggttagggttagggttagggttagggttagggttagggttagggtta

SEQ ID NO: 14 - DNA, 94 bp, artificial
  oligonucleotide
ttagggttagggttagggttagggttagggttagggttagggttagggttagggttaaccctaaccctaaccctaaccctaaccctaaccctaa

SEQ ID NO: 15 - DNA, 35 bp, artificial
  oligonucleotide
ttagggttagggttaaccctaaccctaaaccctaa

SEQ ID NO: 16 - DNA, 34 bp, artificial
  oligonucleotide
ttagggttagggttagggttagggttagggttag

SEQ ID NO: 17 - DNA, 36 bp, artificial
  oligonucleotide
ccctaaccctaaccctaaccctaaccctaaccctaa

SEQ ID NO: 18 - DNA, 35 bp, artificial
  oligonucleotide
ccctaaccctaaccctaaccctaaccctaacccta

SEQ ID NO: 19 - DNA, 72 bp, artificial
  oligonucleotide
ccctaaccctaaccctaaccctaaccctaaccctagggttagggttagggttagggttagggttagggttag

SEQ ID NO: 20 - DNA, 44 bp, artificial
  oligonucleotide
ccctaaccctaaccctaaccctagggttagggttagggttaggg

SEQ ID NO: 21 - DNA, 21 bp, artificial
  oligonucleotide
tagggttagggttagggttag

SEQ ID NO: 22 - DNA, 15 bp, artificial
  oligonucleotide
ctaaccctaacccta

SEQ ID NO: 23 - DNA, 27 bp, artificial
  oligonucleotide
tagggttagggttagggttagggttag

SEQ ID NO: 24 - DNA, 21 bp, artificial
  oligonucleotide
ctaaccctaaccctaacccta

SEQ ID NO: 25 - DNA, 25 bp, artificial
  oligonucleotide
gggttagggttagggttagggttag

SEQ ID NO: 26 - DNA, 46 bp, artificial
  oligonucleotide
gggttagggttagggttagggttagctaaccctaaccctaacccta

SEQ ID NO: 27 - DNA, 46 bp, artificial
  oligonucleotide
gggttagggttagggttagctaaccctaaccctaaccctaacccta

SEQ ID NO: 28 - DNA, 46 bp, artificial
  oligonucleotide
ctaaccctaaccctaaccctagggttagggttagggttagggttag